European Patent Application EP 4 417 974 A1, published August 21, 2024. Title: CD33 as biomarker of HIV control. Applicant: FUNDACIÓ PRIVADA INSTITUT DE RECERCA DE LA SIDA-CAIXA. The sequence listing filed with the application follows.

SEQUENCE LISTING (3 sequences)

SEQ ID NO: 1 - DNA, 18 bp, Human immunodeficiency virus 1
  source 1..18: mol_type = genomic DNA
gacgcaggactcggcttg

SEQ ID NO: 2 - DNA, 18 bp, Human immunodeficiency virus 1
  source 1..18: mol_type = genomic DNA
actgacgctctcgcaccc

SEQ ID NO: 3 - DNA, 23 bp, Human immunodeficiency virus 1
  source 1..23: mol_type = genomic DNA
tttggcgtactcaccagtcgccg